European Patent Specification EP 3 768 302 B1, published May 7, 2025. Title: INTESTINAL ALKALINE PHOSPHATASE FORMULATIONS. Applicant: Synthetic Biologics, Inc. Bristol, Andrew Stapleton, Ray Kaleko, Michael Furlan Freguia, Christian Hubert, Steven Freire, Cristina Gubbins, James. The sequence listing filed with the application follows.

SEQUENCE LISTING (37 sequences)

SEQ ID NO: 1 - protein, 528 aa, Artificial Sequence
  Synthetic polymer
MQGPWVLLLLGLRLQLSLGVIPAEEENPAFWNRQAAEALDAAKKLQPIQKVAKNLILFLGDGLGVPTVTATRILKGQKNGKLGPETPLAMDRFPYLALSKTYNVDRQVPDSAATATAYLCGVKANFQTIGLSAAARFNQCNTTRGNEVISVMNRAKQAGKSVGVVTTTRVQHASPAGTYAHTVNRNWYSDADMPASARQEGCQDIATQLISNMDIDVILGGGRKYMFPMGTPDPEYPADASQNGIRLDGKNLVQEWLAKHQGAWYVWNRTELMQASLDQSVTHLMGLFEPGDTKYEIHRDPTLDPSLMEMTEAALRLLSRNPRGFYLFVEGGRIDHGHHEGVAYQALTEAVMFDDAIERAGQLTSEEDTLTLVTADHSHVFSFGGYTLRGSSIFGLAPSKAQDSKAYTSILYGNGPGYVFNSGVRPDVNESESGSPDYQQQAAVPLSSETHGGEDVAVFARGPQAHLVHGVQEQSFVAHVMAFAACLEPYTACDLAPPACTTDAAHPVAASLPLLAGTLLLLGASAAP

SEQ ID NO: 2 - protein, 533 aa, Artificial Sequence
  Synthetic polymer
MQGACVLLLLGLHLQLSLGLIPAEEENPAFWNRQAAQALDVAKKLQPIQTAAKNVILFLGDGMGVPTVTATRILKGQMNGKLGPETPLAMDQFPYVALSKTYNVDRQVPDSAGTATAYLCGVKGNYRTIGVSAAARYNQCNTTRGNEVTSVINRAKKAGKAVGVVTTTRVQHASPAGAYAHTVNRNWYSDADLPADAQKNGCQDIAAQLVYNMDIDVILGGGRMYMFPEGTPDPEYPDDASVNGVRKDKQNLVQEWQAKHQGAQYVWNRTALLQAADDSSVTHLMGLFEPADMKYNVQQDHTKDPTLAEMTEAALQVLSRNPRGFYLFVEGGRIDHGHHDGKAYMALTEAIMFDNAIAKANELTSELDTLILVTADHSHVFSFGGYTLRGTSIFGLAPGKALDSKSYTSILYGNGPGYALGGGSRPDVNGSTSEEPSYRQQAAVPLASETHGGEDVAVFARGPQAHLVHGVQEETFVAHIMAFAGCVEPYTDCNLPAPATATSIPDAAHLAASPPPLALLAGAMLLLLAPTLY

SEQ ID NO: 3 - protein, 530 aa, Artificial Sequence
  Synthetic polymer
MQWACVLLLLGLWLQLSLTFIPAEEEDPAFWNRQAAQALDVAKKLQPIQTAAKNVILFLGDGMGVPTVTATRILKGQMNGKLGPETPLAMDQFPYVALSKTYNVDRQVPDSAGTATAYLCGVKGNYKTIGVSAAARYNQCNTTSGNEVTSVMNRAKKAGKSVGVVTTSRVQHASPAGAYAHTVNRNWYSDADLPADAQTYGCQDIATQLVNNMDIDVILGGGRMYMFPEGTPDPEYPYDVNQTGVRKDKRNLVQEWQAKHQGAQYVWNRTELLQAANDPSVTHLMGLFEPADMKYNVQQDPTKDPTLEEMTEAALQVLSRNPQGFYLFVEGGRIDHGHHEGKAYMALTDTVMFDNAIAKANELTSELDTLILATADHSHVFSFGGYTLRGTSIFGLAPSKASDNKSYTSILYGNGPGYVLGGGLRPDVNDSISEDPSYRQQAAVPLSSESHGGEDVAVFARGPQAHLVHGVQEETFVAHVMAFAGCVEPYTDCNLPAPSGLSDAAHLAASPPSLALLAGAMLLLLAPALY

SEQ ID NO: 4 - protein, 503 aa, Artificial Sequence
  Synthetic polymer
MQGPWVLLLLGLRLQLSLGVIPAEEENPAFWNRQAAEALDAAKKLQPIQKVAKNLILFLGDGLGVPTVTATRILKGQKNGKLGPETPLAMDRFPYLALSKTYNVDRQVPDSAATATAYLCGVKANFQTIGLSAAARFNQCNTTRGNEVISVMNRAKQAGKSVGVVTTTRVQHASPAGTYAHTVNRNWYSDADMPASARQEGCQDIATQLISNMDIDVILGGGRKYMFPMGTPDPEYPADASQNGIRLDGKNLVQEWLAKHQGAWYVWNRTELMQASLDQSVTHLMGLFEPGDTKYEIHRDPTLDPSLMEMTEAALRLLSRNPRGFYLFVEGGRIDHGHHEGVAYQALTEAVMFDDAIERAGQLTSEEDTLTLVTADHSHVFSFGGYTLRGSSIFGLAPSKAQDSKAYTSILYGNGPGYVFNSGVRPDVNESESGSPDYQQQAAVPLSSETHGGEDVAVFARGPQAHLVHGVQEQSFVAHVMAFAACLEPYTACDLAPPAGTTD

SEQ ID NO: 5 - protein, 506 aa, Artificial Sequence
  Synthetic polymer
MQGACVLLLLGLHLQLSLGLIPAEEENPAFWNRQAAQALDVAKKLQPIQTAAKNVILFLGDGMGVPTVTATRILKGQMNGKLGPETPLAMDQFPYVALSKTYNVDRQVPDSAGTATAYLCGVKGNYRTIGVSAAARYNQCNTTRGNEVTSVINRAKKAGKAVGVVTTTRVQHASPAGAYAHTVNRNWYSDADLPADAQKNGCQDIAAQLVYNMDIDVILGGGRMYMFPEGTPDPEYPDDASVNGVRKDKQNLVQEWQAKHQGAQYVWNRTALLQAADDSSVTHLMGLFEPADMKYNVQQDHTKDPTLAEMTEAALQVLSRNPRGFYLFVEGGRIDHGHHDGKAYMALTEAIMFDNAIAKANELTSELDTLILVTADHSHVFSFGGYTLRGTSIFGLAPGKALDSKSYTSILYGNGPGYALGGGSRPDVNGSTSEEPSYRQQAAVPLASETHGGEDVAVFARGPQAHLVHGVQEETFVAHIMAFAGCVEPYTDCNLPAPATATSIPD

SEQ ID NO: 6 - protein, 503 aa, Artificial Sequence
  Synthetic polymer
MQWACVLLLLGLWLQLSLTFIPAEEEDPAFWNRQAAQALDVAKKLQPIQTAAKNVILFLGDGMGVPTVTATRILKGQMNGKLGPETPLAMDQFPYVALSKTYNVDRQVPDSAGTATAYLCGVKGNYKTIGVSAAARYNQCNTTSGNEVTSVMNRAKKAGKSVGVVTTSRVQHASPAGAYAHTVNRNWYSDADLPADAQTYGCQDIATQLVNNMDIDVILGGGRMYMFPEGTPDPEYPYDVNQTGVRKDKRNLVQEWQAKHQGAQYVWNRTELLQAANDPSVTHLMGLFEPADMKYNVQQDPTKDPTLEEMTEAALQVLSRNPQGFYLFVEGGRIDHGHHEGKAYMALTDTVMFDNAIAKANELTSELDTLILATADHSHVFSFGGYTLRGTSIFGLAPSKASDNKSYTSILYGNGPGYVLGGGLRPDVNDSISEDPSYRQQAAVPLSSESHGGEDVAVFARGPQAHLVHGVQEETFVAHVMAFAGCVEPYTDCNLPAPSGLSD

SEQ ID NO: 7 - protein, 508 aa, Artificial Sequence
  Synthetic polymer
MQWACVLLLLGLWLQLSLTFIPAEEEDPAFWNRQAAQALDVAKKLQPIQTAAKNVILFLGDGMGVPTVTATRILKGQMNGKLGPETPLAMDQFPYVALSKTYNVDRQVPDSAGTATAYLCGVKGNYKTIGVSAAARYNQCNTTSGNEVTSVMNRAKKAGKSVGVVTTSRVQHASPAGAYAHTVNRNWYSDADLPADAQTYGCQDIATQLVNNMDIDVILGGGRMYMFPEGTPDPEYPYDVNQTGVRKDKRNLVQEWQAKHQGAQYVWNRTELLQAANDPSVTHLMGLFEPADMKYNVQQDPTKDPTLEEMTEAALQVLSRNPQGFYLFVEGGRIDHGHHEGKAYMALTDTVMFDNAIAKANELTSELDTLILATADHSHVFSFGGYTLRGTSIFGLAPSKASDNKSYTSILYGNGPGYVLGGGLRPDVNDSISEDPSYRQQAAVPLSSESHGGEDVAVFARGPQAHLVHGVQEETFVAHVMAFAGCVEPYTDCNLPAPSGLSDAAHLA

SEQ ID NO: 8 - protein, 754 aa, Artificial Sequence
  Synthetic polymer
MQGACVLLLLGLHLQLSLGLIPAEEENPAFWNRQAAQALDVAKKLQPIQTAAKNVILFLGDGMGVPTVTATRILKGQMNGKLGPETPLAMDQFPYVALSKTYNVDRQVPDSAGTATAYLCGVKGNYRTIGVSAAARYNQCNTTRGNEVTSVINRAKKAGKAVGVVTTTRVQHASPAGAYAHTVNRNWYSDADLPADAQKNGCQDIAAQLVYNMDIDVILGGGRMYMFPEGTPDPEYPDDASVNGVRKDKQNLVQEWQAKHQGAQYVWNRTALLQAADDSSVTHLMGLFEPADMKYNVQQDHTKDPTLAEMTEAALQVLSRNPRGFYLFVEGGRIDHGHHDGKAYMALTEAIMFDNAIAKANELTSELDTLILVTADHSHVFSFGGYTLRGTSIFGLAPGKALDSKSYTSILYGNGPGYALGGGSRPDVNGSTSEEPSYRQQAAVPLASETHGGEDVAVFARGPQAHLVHGVQEETFVAHIMAFAGCVEPYTDCNLPAPATATSIPDGGSGGSGGGGSGGGGSEPKSCDKTHTCPPCPAPELLGGPSVFLFPPKPKDTLMISRTPEVTCVVVDVSHEDPQVKFNWYVDGVQVHNAKTKPREQQYNSTYRVVSVLTVLHQNWLDGKEYKCKVSNKALPAPIEKTISKAKGQPREPQVYTLPPSREEMTKNQVSLTCLVKGFYPSDIAVEWESNGQPENNYKTTPPVLDSDGSFFLYSKLTVDKSRWQQGNVFSCSVMHEALHNHYTQKSLSLSPGK

SEQ ID NO: 9 - protein, 751 aa, Artificial Sequence
  Synthetic polymer
MQWACVLLLLGLWLQLSLTFIPAEEEDPAFWNRQAAQALDVAKKLQPIQTAAKNVILFLGDGMGVPTVTATRILKGQMNGKLGPETPLAMDQFPYVALSKTYNVDRQVPDSAGTATAYLCGVKGNYKTIGVSAAARYNQCNTTSGNEVTSVMNRAKKAGKSVGVVTTSRVQHASPAGAYAHTVNRNWYSDADLPADAQTYGCQDIATQLVNNMDIDVILGGGRMYMFPEGTPDPEYPYDVNQTGVRKDKRNLVQEWQAKHQGAQYVWNRTELLQAANDPSVTHLMGLFEPADMKYNVQQDPTKDPTLEEMTEAALQVLSRNPQGFYLFVEGGRIDHGHHEGKAYMALTDTVMFDNAIAKANELTSELDTLILATADHSHVFSFGGYTLRGTSIFGLAPSKASDNKSYTSILYGNGPGYVLGGGLRPDVNDSISEDPSYRQQAAVPLSSESHGGEDVAVFARGPQAHLVHGVQEETFVAHVMAFAGCVEPYTDCNLPAPSGLSDGGSGGSGGGGSGGGGSEPKSCDKTHTCPPCPAPELLGGPSVFLFPPKPKDTLMISRTPEVTCVVVDVSHEDPQVKFNWYVDGVQVHNAKTKPREQQYNSTYRVVSVLTVLHQNWLDGKEYKCKVSNKALPAPIEKTISKAKGQPREPQVYTLPPSREEMTKNQVSLTCLVKGFYPSDIAVEWESNGQPENNYKTTPPVLDSDGSFFLYSKLTVDKSRWQQGNVFSCSVMHEALHNHYTQKSLSLSPGK

SEQ ID NO: 10 - protein, 539 aa, Artificial Sequence
  Synthetic polymer
MQWACVLLLLGLWLQLSLTFIPAEEEDPAFWNRQAAQALDVAKKLQPIQTAAKNVILFLGDGMGVPTVTATRILKGQMNGKLGPETPLAMDQFPYVALSKTYNVDRQVPDSAGTATAYLCGVKGNYKTIGVSAAARYNQCNTTSGNEVTSVMNRAKKAGKSVGVVTTSRVQHASPAGAYAHTVNRNWYSDADLPADAQTYGCQDIATQLVNNMDIDVILGGGRMYMFPEGTPDPEYPYDVNQTGVRKDKRNLVQEWQAKHQGAQYVWNRTELLQAANDPSVTHLMGLFEPADMKYNVQQDPTKDPTLEEMTEAALQVLSRNPQGFYLFVEGGRIDHGHHEGKAYMALTDTVMFDNAIAKANELTSELDTLILATADHSHVFSFGGYTLRGTSIFGLAPSKASDNKSYTSILYGNGPGYVLGGGLRPDVNDSISEDPSYRQQAAVPLSSESHGGEDVAVFARGPQAHLVHGVQEETFVAHVMAFAGCVEPYTDCNLEVLFQGPAPPAGTTDAAHPGRSVVPALLPLRAGTLLLLETATAP

SEQ ID NO: 11 - protein, 534 aa, Artificial Sequence
  Synthetic polymer
MQWACVLLLLGLWLQLSLTFIPAEEEDPAFWNRQAAQALDVAKKLQPIQTAAKNVILFLGDGMGVPTVTATRILKGQMNGKLGPETPLAMDQFPYVALSKTYNVDRQVPDSAGTATAYLCGVKGNYKTIGVSAAARYNQCNTTSGNEVTSVMNRAKKAGKSVGVVTTSRVQHASPAGAYAHTVNRNWYSDADLPADAQTYGCQDIATQLVNNMDIDVILGGGRMYMFPEGTPDPEYPYDVNQTGVRKDKRNLVQEWQAKHQGAQYVWNRTELLQAANDPSVTHLMGLFEPADMKYNVQQDPTKDPTLEEMTEAALQVLSRNPQGFYLFVEGGRIDHGHHEGKAYMALTDTVMFDNAIAKANELTSELDTLILATADHSHVFSFGGYTLRGTSIFGLAPSKASDNKSYTSILYGNGPGYVLGGGLRPDVNDSISEDPSYRQQAAVPLSSESHGGEDVAVFARGPQAHLVHGVQEETFVAHVMAFAGCVEPYTDCNLAPPAGTTDAAHPIEGRSVVPALLPLRAGTLLLLETATAP

SEQ ID NO: 12 - DNA, 1669 bp, Artificial Sequence
  Synthetic polymer
atgcaggggccctgggtgctgctgctgctgggcctgaggctacagctctccctgggcgtcatcccaggtaatgaggctccccaagctgttccacacacagggcaccccctcagccaggctgacctgatctctactctccccctggccagctgaggaggagaacccggccttctggaaccgccaggcagctgaggccctggatgctgccaagaagctgcagcccatccagaaggtcgccaagaacctcatcctcttcctgggcgatgggttgggggtgcccacggtgacagccaccaggatcctaaaggggcagaagaatggcaaactggggcctgagacgcccctggccatggaccgcttcccatacctggctctgtccaagacatacaatgtggacagacaggtgccagacagcgcagccacagccacggcctacctgtgcggggtcaaggccaacttccagaccatcggcttgagtgcagccgcccgctttaaccagtgcaacacgacacgcggcaatgaggtcatctccgtgatgaaccgggccaagcaagcaggaaagtcagtaggagtggtgaccaccacacgggtgcagcacgcctcgccagccggcacctacgcacacacagtgaaccgcaactggtactcagatgctgacatgcctgcctcagcccgccaggaggggtgccaggacatcgccactcagctcatctccaacatggacattgacgtgatccttggcggaggccgcaagtacatgtttcccatggggaccccagaccctgagtacccagctgatgccagccagaatggaatcaggctggacgggaagaacctggtgcaggaatggctggcaaagcaccagggtgcctggtatgtgtggaaccgcactgagctcatgcaggcgtccctggaccagtctgtgacccatctcatgggcctctttgagcccggagacacgaaatatgagatccaccgagaccccacactggacccctccctgatggagatgacagaggctgccctgcgcctgctgagcaggaacccccgcggcttctacctctttgtggagggcggccgcatcgaccatggtcatcatgagggtgtggcttaccaggcactcactgaggcggtcatgttcgacgacgccattgagagggcgggccagctcaccagcgaggaggacacgctgaccctcgtcaccgctgaccactcccatgtcttctcctttggtggctacaccttgcgagggagctccatcttcgggttggcccccagcaaggctcaggacagcaaagcctacacgtccatcctgtacggcaatggcccgggctacgtgttcaactcaggcgtgcgaccagacgtgaatgagagcgagagcgggagccccgattaccagcagcaggcggcggtgcccctgtcgtccgagacccacggaggcgaagacgtggcggtgtttgcgcgcggcccgcaggcgcacctggtgcatggtgtgcaggagcagagcttcgtagcgcatgtcatggccttcgctgcctgtctggagccctacacggcctgcgacctggcgcctcccgcctgcaccaccgacgccgcgcacccagttgccgcgtcgctgccactgctggccgggaccctgctgctgctgggggcgtccgctgctccctga

SEQ ID NO: 13 - DNA, 1671 bp, Artificial Sequence
  Synthetic polymer
atgcaggggccctgggtgctgctgctgctgggcctgaggctacagctctccctgggcgtcatcccagctgaggaggagaacccggccttctggaaccgccaggcagctgaggccctggatgctgccaagaagctgcagcccatccagaaggtcgccaagaacctcatcctcttcctgggcgatgggttgggggtgcccacggtgacagccaccaggatcctaaaggggcagaagaatggcaaactggggcctgagacgcccctggccatggaccgcttcccatacctggctctgtccaagacatacaatgtggacagacaggtgccagacagcgcagccacagccacggcctacctgtgcggggtcaaggccaacttccagaccatcggcttgagtgcagccgcccgctttaaccagtgcaacacgacacgcggcaatgaggtcatctccgtgatgaaccgggccaagcaagcaggaaagtcagtaggagtggtgaccaccacacgggtgcagcacgcctcgccagccggcacctacgcacacacagtgaaccgcaactggtactcagatgctgacatgcctgcctcagcccgccaggaggggtgccaggacatcgccactcagctcatctccaacatggacattgacgtgatccttggcggaggccgcaagtacatgtttcccatggggaccccagaccctgagtacccagctgatgccagccagaatggaatcaggctggacgggaagaacctggtgcaggaatggctggcaaagcaccagggtgcctggtatgtgtggaaccgcactgagctcatgcaggcgtccctggaccagtctgtgacccatctcatgggcctctttgagcccggagacacgaaatatgagatccaccgagaccccacactggacccctccctgatggagatgacagaggctgccctgcgcctgctgagcaggaacccccgcggcttctacctctttgtggagggcggccgcatcgaccatggtcatcatgagggtgtggcttaccaggcactcactgaggcggtcatgttcgacgacgccattgagagggcgggccagctcaccagcgaggaggacacgctgaccctcgtcaccgctgaccactcccatgtcttctcctttggtggctacaccttgcgagggagctccatcttcgggttggcccccagcaaggctcaggacagcaaagcctacacgtccatcctgtacggcaatggcccgggctacgtgttcaactcaggcgtgcgaccagacgtgaatgagagcgagagcgggagccccgattaccagcagcaggcggcggtgcccctgtcgtccgagacccacggaggcgaagacgtggcggtgtttgcgcgcggcccgcaggcgcacctggtgcatggtgtgcaggagcagagcttcgtagcgcatgtcatggccttcgctgcctgtctggagccctacacggcctgcgacctggcgcctcccgcctgcaccaccgacgccgcgcacccagttgccgcgtcgctgccactgctggccgggaccctgctgctgctgggggcgtccgctgctccctgatttactaaaaccttgaaataaaattgtaaaacatcagtttgaaggcctgactctcagggtagttcttttttaattctgggtttt

SEQ ID NO: 14 - DNA, 1672 bp, Artificial Sequence
  Synthetic polymer
atgcagtgggcctgtgtgctgctgctgctgggcctgtggctacagctctccctcaccttcatcccaggtaatcaggcggctcccagcagcccctactcacaggggcggctctaggctgacctgaccaacactctccccttgggcagctgaggaggaagaccccgccttctggaaccgccaggcagcccaggcccttgatgtagccaagaagttgcagccgatccagacagctgccaagaatgtcatcctcttcttgggggatgggatgggggtgcctacggtgacagccactcggatcctaaaggggcagatgaatggtaagctgggacctgagacacccctggccatggaccagttcccatacgtggctctgtccaagacatacaacgtggacagacaggtgccagacagcgcaggcactgccactgcctacctgtgtggggtcaagggcaactacaaaaccattggtgtaagtgcagccgcccgctacaaccagtgcaacacaacaagtggcaatgaggtcacgtctgtgatgaaccgggccaagaaagcaggaaagtcagtgggagtggtgaccacctccagggtgcagcatgcctccccagccggtgcttatgcacacacggtgaaccgaaactggtactcagatgccgacctgcctgccgatgcacagacgtatggctgccaggacatcgccacacaactggtcaacaacatggatattgacgtgatcctgggtggaggccgaatgtacatgtttcctgaggggaccccggatcctgaatacccatacgatgtcaatcagactggagtccggaaggacaagcggaatctggtgcaggagtggcaggccaagcaccagggagcccagtatgtgtggaaccgcacggagctccttcaggcagccaatgaccccagtgtaacacacctcatgggcctctttgagccggcagacatgaagtataatgttcagcaagaccccaccaaggacccgaccctggaggagatgacggaggcggccctgcaagtgctgagcaggaacccccagggcttctacctcttcgtggagggaggccgcattgaccacggtcaccatgaaggcaaagcttatatggcactgactgatacagtcatgtttgacaatgccatcgccaaggctaacgagctcactagcgaactggacacgctgatccttgccactgcagaccactcccatgtcttctcttttggtggctacacactgcgtgggacctccattttcggtctggcccccagcaaggcctcagacaacaagtcctacacctccatcctctatggcaatggccctggctacgtgcttggtgggggcttaaggcccgatgttaatgacagcataagcgaggacccctcgtaccggcagcaggcggccgtgcccctgtctagtgagtcccacgggggcgaggacgtggcggtgttcgcgcgaggcccgcaggcgcacctggtgcacggcgtgcaggaggagaccttcgtggcgcacgtcatggcctttgcgggctgcgtggagccctacaccgactgcaatctgccggccccctctggcctctccgacgccgcgcacctggcggccagcccgccttcgctggcgctgctggccggggcgatgctgctgctgctggcgcctgccttgtactga

SEQ ID NO: 15 - DNA, 1869 bp, Artificial Sequence
  Synthetic polymer
atgcagtgggcctgtgtgctgctgctgctgggcctgtggctacagctctccctcaccttcatcccagctgaggaggaagaccccgccttctggaaccgccaggcagcccaggcccttgatgtagccaagaagttgcagccgatccagacagctgccaagaatgtcatcctcttcttgggggatgggatgggggtgcctacggtgacagccactcggatcctaaaggggcagatgaatggtaagctgggacctgagacacccctggccatggaccagttcccatacgtggctctgtccaagacatacaacgtggacagacaggtgccagacagcgcaggcactgccactgcctacctgtgtggggtcaagggcaactacaaaaccattggtgtaagtgcagccgcccgctacaaccagtgcaacacaacaagtggcaatgaggtcacgtctgtgatgaaccgggccaagaaagcaggaaagtcagtgggagtggtgaccacctccagggtgcagcatgcctccccagccggtgcttatgcacacacggtgaaccgaaactggtactcagatgccgacctgcctgccgatgcacagacgtatggctgccaggacatcgccacacaactggtcaacaacatggatattgacgtgatcctgggtggaggccgaatgtacatgtttcctgaggggaccccggatcctgaatacccatacgatgtcaatcagactggagtccggaaggacaagcggaatctggtgcaggagtggcaggccaagcaccagggagcccagtatgtgtggaaccgcacggagctccttcaggcagccaatgaccccagtgtaacacacctcatgggcctctttgagccggcagacatgaagtataatgttcagcaagaccccaccaaggacccgaccctggaggagatgacggaggcggccctgcaagtgctgagcaggaacccccagggcttctacctcttcgtggagggaggccgcattgaccacggtcaccatgaaggcaaagcttatatggcactgactgatacagtcatgtttgacaatgccatcgccaaggctaacgagctcactagcgaactggacacgctgatccttgccactgcagaccactcccatgtcttctcttttggtggctacacactgcgtgggacctccattttcggtctggcccccagcaaggcctcagacaacaagtcctacacctccatcctctatggcaatggccctggctacgtgcttggtgggggcttaaggcccgatgttaatgacagcataagcgaggacccctcgtaccggcagcaggcggccgtgcccctgtctagtgagtcccacgggggcgaggacgtggcggtgttcgcgcgaggcccgcaggcgcacctggtgcacggcgtgcaggaggagaccttcgtggcgcacgtcatggcctttgcgggctgcgtggagccctacaccgactgcaatctgccggccccctctggcctctccgacgccgcgcacctggcggccagcccgccttcgctggcgctgctggccggggcgatgctgctgctgctggcgcctgccttgtactgaggggacccgggggtggggacacaggccccgccctccctgggaggcaggaagcagctctcaaataaactgttctaagtatgatacaggagtgatacatgtgtgaagagaagcccttaggtgggggcacagagtgtctgggtgaggggggtcagggtcacatcaggaggttagggaggggttgatgaagggctgacgttgagcaaagaccaaaggcaactcagaaggacagtggtgcaggactgggtgtggtcagcagggggactggttgggggatcc

SEQ ID NO: 16 - DNA, 1259 bp, Artificial Sequence
  Synthetic polymer
aaaaaacaagacaaagctgagatcagaaatgtcattgtgatgataggcgacggcatggggacgccttacataagagcctaccgttccatgaaaaataacggtgacacaccgaataacccgaagttaacagaatttgaccggaacctgacaggcatgatgatgacgcatccggatgaccctgactataatattacagattcagcagcagccggaacagcattagcgacaggcgttaagacatataacaatgcaattggcgtcgataaaaacggaaaaaaagtgaaatctgtacttgaagaggccaaacagcaaggcaagtcaacagggcttgtcgccacgtctgaaattaaccacgccactccagccgcatatggcgcccacaatgaatcacggaaaaacatggaccaaatcgccaacagctatatggatgacaagataaaaggcaaacataaaatagacgtgctgctcggcggcggaaaatcttattttaaccgcaagaacagaaacttgacaaaggaattcaaacaagccggctacagctatgtgacaactaaacaagcattgaaaaaaaataaagatcagcaggtgctcgggcttttcgcagatggagggcttgctaaagcgctcgaccgtgacagtaaaacaccgtctctcaaagacatgacggtttcagcaattgatcgcctgaaccaaaataaaaaaggatttttcttgatggtcgaagggagccagattgactgggcggcccatgacaatgatacagtaggagccatgagcgaggttaaagattttgaacaggcctataaagccgcgattgaatttgcgaaaaaagacaaacatacacttgtgattgcaactgctgaccatacaaccggcggctttaccattggcgcaaacggggaaaagaattggcacgcagaaccgattctctccgctaagaaaacacctgaattcatggccaaaaaaatcaggaaggcaagccggttaaagatgtgctcgcccgctatgccaatctgaaagtcacatctgaagaaatcaaaagcgttgaagcagctgcacaggctgacaaaagcaaaggggcctccaaagccatcatcaagatttttaatacccgctccaacagcggatggacgagtaccgatcataccggcgaagaagtaccggtatacgcgtacggccccggaaaagaaaaattccgcggattgattaacaatacggaccaggcaaacatcatatttaagattttaaaaactggaaaa

SEQ ID NO: 17 - protein, 420 aa, Artificial Sequence
  Synthetic polymer
KKQDKAEIRNVIVMIGDGMGTPYIRAYRSMKNNGDTPNNPKLTEFDRNLTGMMMTHPDDPDYNITDSAAAGTALATGVKTYNNAIGVDKNGKKVKSVLEEAKQQGKSTGLVATSEINHATPAAYGAHNESRKNMDQIANSYMDDKIKGKHKIDVLLGGGKSYFNRKNRNLTKEFKQAGYSYVTTKQALKKNKDQQVLGLFADGGLAKALDRDSKTPSLKDMTVSAIDRLNQNKKGFFLMVEGSQIDWAAHDNDTVGAMSEVKDFEQAYKAAIEFAKKDKHTLVIATADHTTGGFTIGANGEKNWHAEPILSAKKTPEFMAKKISEGKPVKDVLARYANLKVTSEEIKSVEAAAQADKSKGASKAIIKIFNTRSNSGWTSTDHTGEEVPVYAYGPGKEKFRGLINNTDQANIIFKILKTGK

SEQ ID NO: 18 - protein, 16 aa, Artificial Sequence
  Synthetic polymer
GGSGGSGGGGSGGGGS

SEQ ID NO: 19 - protein, 5 aa, Artificial Sequence
  Synthetic polymer
GGGGS

SEQ ID NO: 20 - protein, 10 aa, Artificial Sequence
  Synthetic polymer
GGGGSGGGGS

SEQ ID NO: 21 - protein, 15 aa, Artificial Sequence
  Synthetic polymer
GGGGSGGGGSGGGGS

SEQ ID NO: 22 - protein, 20 aa, Artificial Sequence
  Synthetic polymer
GGGGSGGGGSGGGGSGGGGS

SEQ ID NO: 23 - protein, 8 aa, Artificial Sequence
  Synthetic polymer
GGGGGGGG

SEQ ID NO: 24 - protein, 6 aa, Artificial Sequence
  Synthetic polymer
GGGGGG

SEQ ID NO: 25 - protein, 5 aa, Artificial Sequence
  Synthetic polymer
EAAAK

SEQ ID NO: 26 - protein, 10 aa, Artificial Sequence
  Synthetic polymer
EAAAKEAAAK

SEQ ID NO: 27 - protein, 15 aa, Artificial Sequence
  Synthetic polymer
EAAAKEAAAKEAAAK

SEQ ID NO: 28 - protein, 12 aa, Artificial Sequence
  Synthetic polymer
AEAAAKEAAAKA

SEQ ID NO: 29 - protein, 17 aa, Artificial Sequence
  Synthetic polymer
AEAAAKEAAAKEAAAKA

SEQ ID NO: 30 - protein, 22 aa, Artificial Sequence
  Synthetic polymer
AEAAAKEAAAKEAAAKEAAAKA

SEQ ID NO: 31 - protein, 27 aa, Artificial Sequence
  Synthetic polymer
AEAAAKEAAAKEAAAKEAAAKEAAAKA

SEQ ID NO: 32 - protein, 12 aa, Artificial Sequence
  Synthetic polymer
AEAAAKEAAAKA

SEQ ID NO: 33 - protein, 46 aa, Artificial Sequence
  Synthetic polymer
AEAAAKEAAAKEAAAKEAAAKALEAEAAAKEAAAKEAAAKEAAAKA

SEQ ID NO: 34 - protein, 5 aa, Artificial Sequence
  Synthetic polymer
PAPAP

SEQ ID NO: 35 - protein, 18 aa, Artificial Sequence
  Synthetic polymer
KESGSVSSEQLAQFRSLD

SEQ ID NO: 36 - protein, 14 aa, Artificial Sequence
  Synthetic polymer
EGKSSGSGSESKST

SEQ ID NO: 37 - protein, 12 aa, Artificial Sequence
  Synthetic polymer
GSAGSAAGSGEF